European Patent Application EP 4 814 014 A1, published September 30, 2026. Title: 结合分子及抗体药物偶联物和用途. Applicant: VelaVigo Bio Inc. The sequence listing filed with the application follows.

SEQUENCE LISTING (138 sequences)

SEQ ID NO: 1 - protein, 117 aa, synthetic construct
AVQLVDSGGGLVQPGGSLRLDCSASGTIIGTYTMAWYRQAPGKQREMVAIITPGGGSHHADSVKGRFTISRDNGKSTVYLQMSSLKFEDTAVYYCNAKARWGTTEYWGQGTQVTVSS

SEQ ID NO: 2 - DNA, 351 bp, synthetic construct
  source 1..351: mol_type = other DNA
gccgtgcagctggtggattctgggggaggcttggtgcagcctggggggtctctgagactcgactgttcagcctctggaaccatcatcggcacctataccatggcctggtaccgccaggctccagggaagcagcgcgagatggtcgcaattattacgcctggtggtggctcacaccatgcagactccgtgaagggccgattcaccatctccagagacaacggcaagtctacggtgtatctccaaatgagcagcctgaaattcgaggacacggccgtctattactgtaatgccaaggcccgttggggcactactgagtactggggccaggggacccaggtcaccgtctcctca

SEQ ID NO: 3 - protein, 5 aa, synthetic construct
TYTMA

SEQ ID NO: 4 - protein, 16 aa, synthetic construct
IITPGGGSHHADSVKG

SEQ ID NO: 5 - protein, 9 aa, synthetic construct
KARWGTTEY

SEQ ID NO: 6 - protein, 126 aa, synthetic construct
QVQLVESGGGLVQPGGSLRLSCAASGLTFSYYAMAWFRQAPGKEREFVAAINWNGGNTYNTDSVKGRFTISRDNAKNTVYLQMNSLKPEDTAVYYCAVRYNSASYLVARSSDYNYWGQGTLVTVSS

SEQ ID NO: 7 - DNA, 378 bp, synthetic construct
  source 1..378: mol_type = other DNA
caggtgcagctggtagagtctgggggaggcttggtgcaacctgggggctctctgagactctcctgtgcagcctctggactcaccttcagttactatgccatggcctggttccgccaggctccagggaaggagcgtgagtttgtagcagctattaactggaatggtggtaacacatacaatacagactccgtgaagggccgattcaccatctccagagacaacgccaagaatacggtgtatctgcaaatgaacagcctgaaacctgaggacacggccgtttattactgtgcagttagatacaatagtgctagttacttagtcgcgagatcgtcagattataactactggggccaggggaccctggtcaccgtctcctca

SEQ ID NO: 8 - protein, 5 aa, synthetic construct
YYAMA

SEQ ID NO: 9 - protein, 17 aa, synthetic construct
AINWNGGNTYNTDSVKG

SEQ ID NO: 10 - protein, 17 aa, synthetic construct
RYNSASYLVARSSDYNY

SEQ ID NO: 11 - protein, 123 aa, synthetic construct
QVQLVESGGGLVQAGGSLRLSCAASGRTGSLHAMGWFRQAPGKERERVATLNLSDGSAVTADSVKGRFTISTDNTKNSVYLQMNSLKPEDTAVYYCTASRSPSGIRYYKPDYWGQGTQVTVSS

SEQ ID NO: 12 - DNA, 369 bp, synthetic construct
  source 1..369: mol_type = other DNA
caggtgcagctggtagaatctgggggaggattggtgcaggctgggggctctctgagactctcctgtgcagcctctggacgcaccggcagtctacatgccatgggctggttccgccaggctccagggaaggagcgtgaaagagtagcaacgcttaacctaagtgatggtagcgcagttactgcagattccgtgaagggccgattcaccatctccacggacaacaccaagaactcggtgtatctgcaaatgaacagcctgaaacctgaggacacggccgtttattactgtacagcgtctcgttccccctcgggtattagatactataagcctgactactggggccaggggacccaggtcaccgtttcctcg

SEQ ID NO: 13 - protein, 5 aa, synthetic construct
LHAMG

SEQ ID NO: 14 - protein, 17 aa, synthetic construct
TLNLSDGSAVTADSVKG

SEQ ID NO: 15 - protein, 14 aa, synthetic construct
SRSPSGIRYYKPDY

SEQ ID NO: 16 - protein, 117 aa, synthetic construct
EVQLVESGGGLVQAGGSLRLSCVASGNIFSSNHMGWFRQAPGKQREFIAYITTREITNYADSVKGRFTISRDNTKNTVYLQMNVLKPEDTAVYYCIADQSREIRRSWGQGTQVTVSS

SEQ ID NO: 17 - DNA, 351 bp, synthetic construct
  source 1..351: mol_type = other DNA
gaggtgcagctggtggagtctgggggaggcttggtgcaggctggggggtctctgagactctcctgtgtagcctctggaaacatcttcagtagcaatcacatgggctggttccgccaggctccagggaagcagcgcgagttcatcgcatatattactactcgtgaaatcacaaactatgcagactccgtgaagggccgattcaccatctccagagacaacaccaagaacacggtgtatctgcaaatgaacgtactgaaacctgaggacacagccgtctattactgtatagcagatcaatctagagaaatccgccgttcctggggccaggggacccaggtcaccgtctcctcg

SEQ ID NO: 18 - protein, 5 aa, synthetic construct
SNHMG

SEQ ID NO: 19 - protein, 16 aa, synthetic construct
YITTREITNYADSVKG

SEQ ID NO: 20 - protein, 9 aa, synthetic construct
DQSREIRRS

SEQ ID NO: 21 - protein, 117 aa, synthetic construct
QSQLAESGGGLVQSGGSLGLSCVASGFTISRSIMSWYRQPPGKERDWVASIGSAGNTNYVDSVKGRFTISRDVAKNTVYLQMNSLKPEDTAVYYCKTTLAVSFSEYWGQGTQVTVSS

SEQ ID NO: 22 - DNA, 351 bp, synthetic construct
  source 1..351: mol_type = other DNA
caaagccagctggccgaaagcggcggcggactggtgcagagcggaggatctctgggcctgtcttgtgtggcttctggctttacaatcagccggtccatcatgagctggtatagacagcctcctggcaaggaacgggactgggtcgccagcatcggcagcgccggcaatacaaactacgtggacagcgtgaaaggcagattcaccatctccagagatgtggccaagaacaccgtgtacctgcagatgaacagcctgaagcccgaggacaccgccgtgtactactgcaagaccaccctggctgtgtccttcagcgagtactggggccagggcacacaggtgaccgtttctagc

SEQ ID NO: 23 - protein, 5 aa, synthetic construct
RSIMS

SEQ ID NO: 24 - protein, 16 aa, synthetic construct
SIGSAGNTNYVDSVKG

SEQ ID NO: 25 - protein, 9 aa, synthetic construct
TLAVSFSEY

SEQ ID NO: 26 - protein, 117 aa, synthetic construct
QVQLVESGGGLVQPGGSLRLSCEASGFTFSSYVMSWYRQAPGKERELVALISSTTGSSTKYGDSVKGRFTISRDNAKNTVYLQMNSLKPEDTAVYYCNAMIGWNNHWGQGTHVTVSS

SEQ ID NO: 27 - DNA, 351 bp, synthetic construct
  source 1..351: mol_type = other DNA
caagtgcagctggtggaaagcggcggcggactggttcagcctggaggatctctcagactgagctgcgaggccagcggctttaccttcagctcctacgtgatgagctggtatagacaggcccctggcaaagagcgggaactggtcgccctgatctctagcaccaccggcagctctacaaagtacggcgatagcgtgaagggcagattcacaatcagccgggacaacgccaagaacaccgtgtacctgcagatgaacagcctgaagcccgaggacaccgccgtgtactactgtaatgctatgatcggctggaacaaccactggggccagggcacccacgtgacagtgtcctcc

SEQ ID NO: 28 - protein, 5 aa, synthetic construct
SYVMS

SEQ ID NO: 29 - protein, 18 aa, synthetic construct
LISSTTGSSTKYGDSVKG

SEQ ID NO: 30 - protein, 7 aa, synthetic construct
MIGWNNH

SEQ ID NO: 31 - protein, 117 aa, synthetic construct
EVQLVESGGGLVQPGGSLRLSCSASGTIIGTYTMAWYRQAPGKQREMVAIITPGGGSHHADSVKGRFTISRDNSKNTLYLQMSSLRAEDTAVYYCNAKARWGTTEYWGQGTLVTVSS

SEQ ID NO: 32 - protein, 126 aa, synthetic construct
EVQLLESGGGLVQPGGSLRLSCAASGLTFSYYAMAWFRQAPGKEREFVAAINWNQGNTYNTDSVKGRFTISRDNSKNTVYLQMNSLTPEDTAVYYCAVRYNQASYLVARSSDYNYWGQGTLVTVSS

SEQ ID NO: 33 - DNA, 378 bp, synthetic construct
  source 1..378: mol_type = other DNA
gaagtgcagctgctcgagtccgggggcgggctggtgcagcccggcggcagcctcagactgagctgcgccgctagcggcctgaccttcagctactacgccatggcctggttcagacaagcccccggcaaggagagagagttcgtggccgccatcaactggaaccaaggcaacacctacaacaccgacagcgtgaagggcagattcaccatcagcagagacaacagcaagaacaccgtgtacctgcagatgaacagcctgacccccgaggacaccgccgtgtactactgcgccgtgagatacaaccaagctagctacctggtggctagaagcagcgactacaactactggggccaaggcaccctggtgaccgtgagcagc

SEQ ID NO: 34 - protein, 17 aa, synthetic construct
AINWNQGNTYNTDSVKG

SEQ ID NO: 35 - protein, 17 aa, synthetic construct
RYNQASYLVARSSDYNY

SEQ ID NO: 36 - protein, 123 aa, synthetic construct
QVQLVESGGGLVQPGGSLRLSCAASGRTGSLHAMGWFRQAPGKERERVATLRLSDVSAVTADSVKGRFTISTDNSKNTLYLQMNSLRAEDTAVYYCTASRSPSGIRYYKPDYWGQGTLVTVSS

SEQ ID NO: 37 - DNA, 369 bp, synthetic construct
  source 1..369: mol_type = other DNA
caggtgcagctcgtggaatcaggaggtggactggtgcagccaggtggatctctgaggctgtcttgtgcagctagcggaagaacaggctctctgcacgccatgggttggttcagacaggctccaggcaaggagagagaaagagtggccacactgcggctgagcgacgtgtcagcagtgacagcagacagcgtgaagggtagattcaccatcagtaccgacaacagcaagaacaccctgtacctgcagatgaacagcctgagagctgaggataccgcagtgtactattgcaccgcttctcgaagccctagcggcattcggtactacaagcctgactattggggtcaaggcacactggtcacagtgtcatct

SEQ ID NO: 38 - protein, 17 aa, synthetic construct
TLRLSDVSAVTADSVKG

SEQ ID NO: 39 - protein, 117 aa, synthetic construct
EVQLVESGGGLVQPGGSLRLSCTASGNIFSSYHMGWFRQAPGKQREFIAYITTREITNYADSVKGRFTISRDNSKNTLYLQMNSLRAEDTAVYYCIADQSREIRRSWGQGTLVTVSS

SEQ ID NO: 40 - protein, 117 aa, synthetic construct
EVQLVESGGGLIQAGGSLRLSCTASGNIFSSYHMGWFRQAPGKQREFIAYITTREITNYADSVKGRFTISRDNSKNTVYLQMNNLRSEDTAVYYCIADQSREIRRSWGQGTLVTVSS

SEQ ID NO: 41 - protein, 5 aa, synthetic construct
SYHMG

SEQ ID NO: 42 - protein, 117 aa, synthetic construct
QSQLVESGGGLVKPGGSLRLSCVASGFTISRSIMSWYRQAPGKERDWVASIGSAGNTNYVDSVKGRFTISRDNAKNSLYLQMNSLRAEDTAVYYCKTTLAVSFSEYWGQGTLVTVSS

SEQ ID NO: 43 - protein, 5 aa, synthetic construct
GGGGS

SEQ ID NO: 44 - protein, 10 aa, synthetic construct
GGGGSGGGGS

SEQ ID NO: 45 - protein, 115 aa, synthetic construct [sequence omitted]

SEQ ID NO: 46 - protein, 5 aa, synthetic construct
SFGMS

SEQ ID NO: 47 - protein, 17 aa, synthetic construct
SISGSGSDTLYADSVKG

SEQ ID NO: 48 - protein, 6 aa, synthetic construct
GGSLSR

SEQ ID NO: 49 - protein, 5 aa, synthetic construct
EPKSS

SEQ ID NO: 50 - protein, 5 aa, synthetic construct
EPKSC

SEQ ID NO: 51 - protein, 366 aa, synthetic construct
AVQLVDSGGGLVQPGGSLRLDCSASGTIIGTYTMAWYRQAPGKQREMVAIITPGGGSHHADSVKGRFTISRDNGKSTVYLQMSSLKFEDTAVYYCNAKARWGTTEYWGQGTQVTVSSGGGGSQSQLAESGGGLVQSGGSLGLSCVASGFTISRSIMSWYRQPPGKERDWVASIGSAGNTNYVDSVKGRFTISRDVAKNTVYLQMNSLKPEDTAVYYCKTTLAVSFSEYWGQGTQVTVSSGGGGSGGGGSEVQLVESGGGLVQAGGSLRLSCVASGNIFSSNHMGWFRQAPGKQREFIAYITTREITNYADSVKGRFTISRDNTKNTVYLQMNVLKPEDTAVYYCIADQSREIRRSWGQGTQVTVSS

SEQ ID NO: 52 - protein, 366 aa, synthetic construct
AVQLVDSGGGLVQPGGSLRLDCSASGTIIGTYTMAWYRQAPGKQREMVAIITPGGGSHHADSVKGRFTISRDNGKSTVYLQMSSLKFEDTAVYYCNAKARWGTTEYWGQGTQVTVSSGGGGSEVQLVESGGGLVQAGGSLRLSCVASGNIFSSNHMGWFRQAPGKQREFIAYITTREITNYADSVKGRFTISRDNTKNTVYLQMNVLKPEDTAVYYCIADQSREIRRSWGQGTQVTVSSGGGGSGGGGSQSQLAESGGGLVQSGGSLGLSCVASGFTISRSIMSWYRQPPGKERDWVASIGSAGNTNYVDSVKGRFTISRDVAKNTVYLQMNSLKPEDTAVYYCKTTLAVSFSEYWGQGTQVTVSS

SEQ ID NO: 53 - protein, 375 aa, synthetic construct
QVQLVESGGGLVQPGGSLRLSCAASGLTFSYYAMAWFRQAPGKEREFVAAINWNGGNTYNTDSVKGRFTISRDNAKNTVYLQMNSLKPEDTAVYYCAVRYNSASYLVARSSDYNYWGQGTLVTVSSGGGGSQSQLAESGGGLVQSGGSLGLSCVASGFTISRSIMSWYRQPPGKERDWVASIGSAGNTNYVDSVKGRFTISRDVAKNTVYLQMNSLKPEDTAVYYCKTTLAVSFSEYWGQGTQVTVSSGGGGSGGGGSEVQLVESGGGLVQAGGSLRLSCVASGNIFSSNHMGWFRQAPGKQREFIAYITTREITNYADSVKGRFTISRDNTKNTVYLQMNVLKPEDTAVYYCIADQSREIRRSWGQGTQVTVSS

SEQ ID NO: 54 - protein, 375 aa, synthetic construct
QVQLVESGGGLVQPGGSLRLSCAASGLTFSYYAMAWFRQAPGKEREFVAAINWNGGNTYNTDSVKGRFTISRDNAKNTVYLQMNSLKPEDTAVYYCAVRYNSASYLVARSSDYNYWGQGTLVTVSSGGGGSEVQLVESGGGLVQAGGSLRLSCVASGNIFSSNHMGWFRQAPGKQREFIAYITTREITNYADSVKGRFTISRDNTKNTVYLQMNVLKPEDTAVYYCIADQSREIRRSWGQGTQVTVSSGGGGSGGGGSQSQLAESGGGLVQSGGSLGLSCVASGFTISRSIMSWYRQPPGKERDWVASIGSAGNTNYVDSVKGRFTISRDVAKNTVYLQMNSLKPEDTAVYYCKTTLAVSFSEYWGQGTQVTVSS

SEQ ID NO: 55 - protein, 372 aa, synthetic construct
QVQLVESGGGLVQAGGSLRLSCAASGRTGSLHAMGWFRQAPGKERERVATLNLSDGSAVTADSVKGRFTISTDNTKNSVYLQMNSLKPEDTAVYYCTASRSPSGIRYYKPDYWGQGTQVTVSSGGGGSQSQLAESGGGLVQSGGSLGLSCVASGFTISRSIMSWYRQPPGKERDWVASIGSAGNTNYVDSVKGRFTISRDVAKNTVYLQMNSLKPEDTAVYYCKTTLAVSFSEYWGQGTQVTVSSGGGGSGGGGSEVQLVESGGGLVQAGGSLRLSCVASGNIFSSNHMGWFRQAPGKQREFIAYITTREITNYADSVKGRFTISRDNTKNTVYLQMNVLKPEDTAVYYCIADQSREIRRSWGQGTQVTVSS

SEQ ID NO: 56 - protein, 372 aa, synthetic construct
QVQLVESGGGLVQAGGSLRLSCAASGRTGSLHAMGWFRQAPGKERERVATLNLSDGSAVTADSVKGRFTISTDNTKNSVYLQMNSLKPEDTAVYYCTASRSPSGIRYYKPDYWGQGTQVTVSSGGGGSEVQLVESGGGLVQAGGSLRLSCVASGNIFSSNHMGWFRQAPGKQREFIAYITTREITNYADSVKGRFTISRDNTKNTVYLQMNVLKPEDTAVYYCIADQSREIRRSWGQGTQVTVSSGGGGSGGGGSQSQLAESGGGLVQSGGSLGLSCVASGFTISRSIMSWYRQPPGKERDWVASIGSAGNTNYVDSVKGRFTISRDVAKNTVYLQMNSLKPEDTAVYYCKTTLAVSFSEYWGQGTQVTVSS

SEQ ID NO: 57 - protein, 372 aa, synthetic construct
QVQLVESGGGLVQPGGSLRLSCAASGRTGSLHAMGWFRQAPGKERERVATLRLSDVSAVTADSVKGRFTISTDNSKNTLYLQMNSLRAEDTAVYYCTASRSPSGIRYYKPDYWGQGTLVTVSSGGGGSEVQLVESGGGLVQPGGSLRLSCTASGNIFSSYHMGWFRQAPGKQREFIAYITTREITNYADSVKGRFTISRDNSKNTLYLQMNSLRAEDTAVYYCIADQSREIRRSWGQGTLVTVSSGGGGSGGGGSQSQLAESGGGLVQSGGSLGLSCVASGFTISRSIMSWYRQPPGKERDWVASIGSAGNTNYVDSVKGRFTISRDVAKNTVYLQMNSLKPEDTAVYYCKTTLAVSFSEYWGQGTQVTVSS

SEQ ID NO: 58 - protein, 372 aa, synthetic construct
QVQLVESGGGLVQPGGSLRLSCAASGRTGSLHAMGWFRQAPGKERERVATLRLSDVSAVTADSVKGRFTISTDNSKNTLYLQMNSLRAEDTAVYYCTASRSPSGIRYYKPDYWGQGTLVTVSSGGGGSEVQLVESGGGLVQPGGSLRLSCTASGNIFSSYHMGWFRQAPGKQREFIAYITTREITNYADSVKGRFTISRDNSKNTLYLQMNSLRAEDTAVYYCIADQSREIRRSWGQGTLVTVSSGGGGSGGGGSQSQLVESGGGLVKPGGSLRLSCVASGFTISRSIMSWYRQAPGKERDWVASIGSAGNTNYVDSVKGRFTISRDNAKNSLYLQMNSLRAEDTAVYYCKTTLAVSFSEYWGQGTLVTVSS

SEQ ID NO: 59 - protein, 372 aa, synthetic construct
QVQLVESGGGLVQPGGSLRLSCAASGRTGSLHAMGWFRQAPGKERERVATLRLSDVSAVTADSVKGRFTISTDNSKNTLYLQMNSLRAEDTAVYYCTASRSPSGIRYYKPDYWGQGTLVTVSSGGGGSEVQLVESGGGLVQPGGSLRLSCTASGNIFSSYHMGWFRQAPGKQREFIAYITTREITNYADSVKGRFTISRDNSKNTLYLQMNSLRAEDTAVYYCIADQSREIRRSWGQGTLVTVSSGGGGSGGGGSEVQLVESGGGLVQPGGSLRLSCTASGNIFSSYHMGWFRQAPGKQREFIAYITTREITNYADSVKGRFTISRDNSKNTLYLQMNSLRAEDTAVYYCIADQSREIRRSWGQGTLVTVSS

SEQ ID NO: 60 - protein, 372 aa, synthetic construct
QVQLVESGGGLVQPGGSLRLSCAASGRTGSLHAMGWFRQAPGKERERVATLRLSDVSAVTADSVKGRFTISTDNSKNTLYLQMNSLRAEDTAVYYCTASRSPSGIRYYKPDYWGQGTLVTVSSGGGGSQSQLVESGGGLVKPGGSLRLSCVASGFTISRSIMSWYRQAPGKERDWVASIGSAGNTNYVDSVKGRFTISRDNAKNSLYLQMNSLRAEDTAVYYCKTTLAVSFSEYWGQGTLVTVSSGGGGSGGGGSQSQLVESGGGLVKPGGSLRLSCVASGFTISRSIMSWYRQAPGKERDWVASIGSAGNTNYVDSVKGRFTISRDNAKNSLYLQMNSLRAEDTAVYYCKTTLAVSFSEYWGQGTLVTVSS

SEQ ID NO: 61 - protein, 366 aa, synthetic construct
EVQLVESGGGLVQPGGSLRLSCSASGTIIGTYTMAWYRQAPGKQREMVAIITPGGGSHHADSVKGRFTISRDNSKNTLYLQMSSLRAEDTAVYYCNAKARWGTTEYWGQGTLVTVSSGGGGSEVQLVESGGGLVQPGGSLRLSCTASGNIFSSYHMGWFRQAPGKQREFIAYITTREITNYADSVKGRFTISRDNSKNTLYLQMNSLRAEDTAVYYCIADQSREIRRSWGQGTLVTVSSGGGGSGGGGSQSQLVESGGGLVKPGGSLRLSCVASGFTISRSIMSWYRQAPGKERDWVASIGSAGNTNYVDSVKGRFTISRDNAKNSLYLQMNSLRAEDTAVYYCKTTLAVSFSEYWGQGTLVTVSS

SEQ ID NO: 62 - protein, 366 aa, synthetic construct
EVQLVESGGGLVQPGGSLRLSCSASGTIIGTYTMAWYRQAPGKQREMVAIITPGGGSHHADSVKGRFTISRDNSKNTLYLQMSSLRAEDTAVYYCNAKARWGTTEYWGQGTLVTVSSGGGGSEVQLVESGGGLVQPGGSLRLSCTASGNIFSSYHMGWFRQAPGKQREFIAYITTREITNYADSVKGRFTISRDNSKNTLYLQMNSLRAEDTAVYYCIADQSREIRRSWGQGTLVTVSSGGGGSGGGGSEVQLVESGGGLVQPGGSLRLSCTASGNIFSSYHMGWFRQAPGKQREFIAYITTREITNYADSVKGRFTISRDNSKNTLYLQMNSLRAEDTAVYYCIADQSREIRRSWGQGTLVTVSS

SEQ ID NO: 63 - protein, 366 aa, synthetic construct
EVQLVESGGGLVQPGGSLRLSCSASGTIIGTYTMAWYRQAPGKQREMVAIITPGGGSHHADSVKGRFTISRDNSKNTLYLQMSSLRAEDTAVYYCNAKARWGTTEYWGQGTLVTVSSGGGGSQSQLVESGGGLVKPGGSLRLSCVASGFTISRSIMSWYRQAPGKERDWVASIGSAGNTNYVDSVKGRFTISRDNAKNSLYLQMNSLRAEDTAVYYCKTTLAVSFSEYWGQGTLVTVSSGGGGSGGGGSQSQLVESGGGLVKPGGSLRLSCVASGFTISRSIMSWYRQAPGKERDWVASIGSAGNTNYVDSVKGRFTISRDNAKNSLYLQMNSLRAEDTAVYYCKTTLAVSFSEYWGQGTLVTVSS

SEQ ID NO: 64 - protein, 375 aa, synthetic construct
EVQLLESGGGLVQPGGSLRLSCAASGLTFSYYAMAWFRQAPGKEREFVAAINWNQGNTYNTDSVKGRFTISRDNSKNTVYLQMNSLTPEDTAVYYCAVRYNQASYLVARSSDYNYWGQGTLVTVSSGGGGSEVQLVESGGGLVQPGGSLRLSCTASGNIFSSYHMGWFRQAPGKQREFIAYITTREITNYADSVKGRFTISRDNSKNTLYLQMNSLRAEDTAVYYCIADQSREIRRSWGQGTLVTVSSGGGGSGGGGSQSQLVESGGGLVKPGGSLRLSCVASGFTISRSIMSWYRQAPGKERDWVASIGSAGNTNYVDSVKGRFTISRDNAKNSLYLQMNSLRAEDTAVYYCKTTLAVSFSEYWGQGTLVTVSS

SEQ ID NO: 65 - protein, 375 aa, synthetic construct
EVQLLESGGGLVQPGGSLRLSCAASGLTFSYYAMAWFRQAPGKEREFVAAINWNQGNTYNTDSVKGRFTISRDNSKNTVYLQMNSLTPEDTAVYYCAVRYNQASYLVARSSDYNYWGQGTLVTVSSGGGGSEVQLVESGGGLVQPGGSLRLSCTASGNIFSSYHMGWFRQAPGKQREFIAYITTREITNYADSVKGRFTISRDNSKNTLYLQMNSLRAEDTAVYYCIADQSREIRRSWGQGTLVTVSSGGGGSGGGGSEVQLVESGGGLVQPGGSLRLSCTASGNIFSSYHMGWFRQAPGKQREFIAYITTREITNYADSVKGRFTISRDNSKNTLYLQMNSLRAEDTAVYYCIADQSREIRRSWGQGTLVTVSS

SEQ ID NO: 66 - protein, 375 aa, synthetic construct
EVQLLESGGGLVQPGGSLRLSCAASGLTFSYYAMAWFRQAPGKEREFVAAINWNQGNTYNTDSVKGRFTISRDNSKNTVYLQMNSLTPEDTAVYYCAVRYNQASYLVARSSDYNYWGQGTLVTVSSGGGGSQSQLVESGGGLVKPGGSLRLSCVASGFTISRSIMSWYRQAPGKERDWVASIGSAGNTNYVDSVKGRFTISRDNAKNSLYLQMNSLRAEDTAVYYCKTTLAVSFSEYWGQGTLVTVSSGGGGSGGGGSQSQLVESGGGLVKPGGSLRLSCVASGFTISRSIMSWYRQAPGKERDWVASIGSAGNTNYVDSVKGRFTISRDNAKNSLYLQMNSLRAEDTAVYYCKTTLAVSFSEYWGQGTLVTVSS

SEQ ID NO: 67 - protein, 492 aa, synthetic construct
QVQLVESGGGLVQPGGSLRLSCAASGRTGSLHAMGWFRQAPGKERERVATLRLSDVSAVTADSVKGRFTISTDNSKNTLYLQMNSLRAEDTAVYYCTASRSPSGIRYYKPDYWGQGTLVTVSSGGGGSEVQLVESGGGLVQPGGSLRLSCTASGNIFSSYHMGWFRQAPGKQREFIAYITTREITNYADSVKGRFTISRDNSKNTLYLQMNSLRAEDTAVYYCIADQSREIRRSWGQGTLVTVSSGGGGSGGGGSQSQLAESGGGLVQSGGSLGLSCVASGFTISRSIMSWYRQPPGKERDWVASIGSAGNTNYVDSVKGRFTISRDVAKNTVYLQMNSLKPEDTAVYYCKTTLAVSFSEYWGQGTQVTVSSGGGGSEVQLVESGGGLVQPGNSLRLSCAASGFTFSSFGMSWVRQAPGKGLEWVSSISGSGSDTLYADSVKGRFTISRDNAKTTLYLQMNSLRPEDTAVYYCTIGGSLSRSSQGTLVTVSS

SEQ ID NO: 68 - protein, 492 aa, synthetic construct
QVQLVESGGGLVQPGGSLRLSCAASGRTGSLHAMGWFRQAPGKERERVATLRLSDVSAVTADSVKGRFTISTDNSKNTLYLQMNSLRAEDTAVYYCTASRSPSGIRYYKPDYWGQGTLVTVSSGGGGSEVQLVESGGGLVQPGGSLRLSCTASGNIFSSYHMGWFRQAPGKQREFIAYITTREITNYADSVKGRFTISRDNSKNTLYLQMNSLRAEDTAVYYCIADQSREIRRSWGQGTLVTVSSGGGGSGGGGSQSQLVESGGGLVKPGGSLRLSCVASGFTISRSIMSWYRQAPGKERDWVASIGSAGNTNYVDSVKGRFTISRDNAKNSLYLQMNSLRAEDTAVYYCKTTLAVSFSEYWGQGTLVTVSSGGGGSEVQLVESGGGLVQPGNSLRLSCAASGFTFSSFGMSWVRQAPGKGLEWVSSISGSGSDTLYADSVKGRFTISRDNAKTTLYLQMNSLRPEDTAVYYCTIGGSLSRSSQGTLVTVSS

SEQ ID NO: 69 - protein, 476 aa, synthetic construct
QSQLAESGGGLVQSGGSLGLSCVASGFTISRSIMSWYRQPPGKERDWVASIGSAGNTNYVDSVKGRFTISRDVAKNTVYLQMNSLKPEDTAVYYCKTTLAVSFSEYWGQGTQVTVSSGGGGSGGGGSEVQLVESGGGLVQPGGSLRLSCTASGNIFSSYHMGWFRQAPGKQREFIAYITTREITNYADSVKGRFTISRDNSKNTLYLQMNSLRAEDTAVYYCIADQSREIRRSWGQGTLVTVSSEPKSSDKTHTCPPCPAPEAAGGPSVFLFPPKPKDTLMISRTPEVTCVVVDVSHEDPEVKFNWYVDGVEVHNAKTKPREEQYNSTYRVVSVLTVLHQDWLNGKEYKCKVSNKALPAPIEKTISKAKGQPREPQVYTLPPSRDELTKNQVSLWCLVKGFYPSDIAVEWESNGQPENNYKTTPPVLDSDGSFFLYSKLTVDKSRWQQGNVFSCSVMHEALHNHYTQKSLSLSPGK

SEQ ID NO: 70 - protein, 355 aa, synthetic construct
QVQLVESGGGLVQPGGSLRLSCAASGRTGSLHAMGWFRQAPGKERERVATLRLSDVSAVTADSVKGRFTISTDNSKNTLYLQMNSLRAEDTAVYYCTASRSPSGIRYYKPDYWGQGTLVTVSSEPKSSDKTHTCPPCPAPEAAGGPSVFLFPPKPKDTLMISRTPEVTCVVVDVSHEDPEVKFNWYVDGVEVHNAKTKPREEQYNSTYRVVSVLTVLHQDWLNGKEYKCKVSNKALPAPIEKTISKAKGQPREPQVYTLPPSRDELTKNQVSLSCAVKGFYPSDIAVEWESNGQPENNYKTTPPVLDSDGSFFLVSKLTVDKSRWQQGNVFSCSVMHEALHNHYTQKSLSLSPGK

SEQ ID NO: 71 - protein, 349 aa, synthetic construct
EVQLVESGGGLVQPGGSLRLSCSASGTIIGTYTMAWYRQAPGKQREMVAIITPGGGSHHADSVKGRFTISRDNSKNTLYLQMSSLRAEDTAVYYCNAKARWGTTEYWGQGTLVTVSSEPKSSDKTHTCPPCPAPEAAGGPSVFLFPPKPKDTLMISRTPEVTCVVVDVSHEDPEVKFNWYVDGVEVHNAKTKPREEQYNSTYRVVSVLTVLHQDWLNGKEYKCKVSNKALPAPIEKTISKAKGQPREPQVYTLPPSRDELTKNQVSLSCAVKGFYPSDIAVEWESNGQPENNYKTTPPVLDSDGSFFLVSKLTVDKSRWQQGNVFSCSVMHEALHNHYTQKSLSLSPGK

SEQ ID NO: 72 - protein, 358 aa, synthetic construct
EVQLLESGGGLVQPGGSLRLSCAASGLTFSYYAMAWFRQAPGKEREFVAAINWNQGNTYNTDSVKGRFTISRDNSKNTVYLQMNSLTPEDTAVYYCAVRYNQASYLVARSSDYNYWGQGTLVTVSSEPKSSDKTHTCPPCPAPEAAGGPSVFLFPPKPKDTLMISRTPEVTCVVVDVSHEDPEVKFNWYVDGVEVHNAKTKPREEQYNSTYRVVSVLTVLHQDWLNGKEYKCKVSNKALPAPIEKTISKAKGQPREPQVYTLPPSRDELTKNQVSLSCAVKGFYPSDIAVEWESNGQPENNYKTTPPVLDSDGSFFLVSKLTVDKSRWQQGNVFSCSVMHEALHNHYTQKSLSLSPGK

SEQ ID NO: 73 - protein, 476 aa, synthetic construct
QSQLVESGGGLVKPGGSLRLSCVASGFTISRSIMSWYRQAPGKERDWVASIGSAGNTNYVDSVKGRFTISRDNAKNSLYLQMNSLRAEDTAVYYCKTTLAVSFSEYWGQGTLVTVSSGGGGSGGGGSEVQLVESGGGLVQPGGSLRLSCTASGNIFSSYHMGWFRQAPGKQREFIAYITTREITNYADSVKGRFTISRDNSKNTLYLQMNSLRAEDTAVYYCIADQSREIRRSWGQGTLVTVSSEPKSSDKTHTCPPCPAPEAAGGPSVFLFPPKPKDTLMISRTPEVTCVVVDVSHEDPEVKFNWYVDGVEVHNAKTKPREEQYNSTYRVVSVLTVLHQDWLNGKEYKCKVSNKALPAPIEKTISKAKGQPREPQVYTLPPSRDELTKNQVSLWCLVKGFYPSDIAVEWESNGQPENNYKTTPPVLDSDGSFFLYSKLTVDKSRWQQGNVFSCSVMHEALHNHYTQKSLSLSPGK

SEQ ID NO: 74 - protein, 476 aa, synthetic construct
QSQLVESGGGLVKPGGSLRLSCVASGFTISRSIMSWYRQAPGKERDWVASIGSAGNTNYVDSVKGRFTISRDNAKNSLYLQMNSLRAEDTAVYYCKTTLAVSFSEYWGQGTLVTVSSGGGGSGGGGSQSQLVESGGGLVKPGGSLRLSCVASGFTISRSIMSWYRQAPGKERDWVASIGSAGNTNYVDSVKGRFTISRDNAKNSLYLQMNSLRAEDTAVYYCKTTLAVSFSEYWGQGTLVTVSSEPKSSDKTHTCPPCPAPEAAGGPSVFLFPPKPKDTLMISRTPEVTCVVVDVSHEDPEVKFNWYVDGVEVHNAKTKPREEQYNSTYRVVSVLTVLHQDWLNGKEYKCKVSNKALPAPIEKTISKAKGQPREPQVYTLPPSRDELTKNQVSLWCLVKGFYPSDIAVEWESNGQPENNYKTTPPVLDSDGSFFLYSKLTVDKSRWQQGNVFSCSVMHEALHNHYTQKSLSLSPGK

SEQ ID NO: 75 - protein, 476 aa, synthetic construct
EVQLVESGGGLVQPGGSLRLSCTASGNIFSSYHMGWFRQAPGKQREFIAYITTREITNYADSVKGRFTISRDNSKNTLYLQMNSLRAEDTAVYYCIADQSREIRRSWGQGTLVTVSSGGGGSGGGGSEVQLVESGGGLVQPGGSLRLSCTASGNIFSSYHMGWFRQAPGKQREFIAYITTREITNYADSVKGRFTISRDNSKNTLYLQMNSLRAEDTAVYYCIADQSREIRRSWGQGTLVTVSSEPKSSDKTHTCPPCPAPEAAGGPSVFLFPPKPKDTLMISRTPEVTCVVVDVSHEDPEVKFNWYVDGVEVHNAKTKPREEQYNSTYRVVSVLTVLHQDWLNGKEYKCKVSNKALPAPIEKTISKAKGQPREPQVYTLPPSRDELTKNQVSLWCLVKGFYPSDIAVEWESNGQPENNYKTTPPVLDSDGSFFLYSKLTVDKSRWQQGNVFSCSVMHEALHNHYTQKSLSLSPGK

SEQ ID NO: 76 - protein, 492 aa, synthetic construct
QVQLVESGGGLVQPGGSLRLSCAASGRTGSLHAMGWFRQAPGKERERVATLRLSDVSAVTADSVKGRFTISTDNSKNTLYLQMNSLRAEDTAVYYCTASRSPSGIRYYKPDYWGQGTLVTVSSGGGGSEVQLVESGGGLVQPGGSLRLSCTASGNIFSSYHMGWFRQAPGKQREFIAYITTREITNYADSVKGRFTISRDNSKNTLYLQMNSLRAEDTAVYYCIADQSREIRRSWGQGTLVTVSSGGGGSGGGGSEVQLVESGGGLVQPGGSLRLSCTASGNIFSSYHMGWFRQAPGKQREFIAYITTREITNYADSVKGRFTISRDNSKNTLYLQMNSLRAEDTAVYYCIADQSREIRRSWGQGTLVTVSSGGGGSEVQLVESGGGLVQPGNSLRLSCAASGFTFSSFGMSWVRQAPGKGLEWVSSISGSGSDTLYADSVKGRFTISRDNAKTTLYLQMNSLRPEDTAVYYCTIGGSLSRSSQGTLVTVSS

SEQ ID NO: 77 - protein, 492 aa, synthetic construct
QVQLVESGGGLVQPGGSLRLSCAASGRTGSLHAMGWFRQAPGKERERVATLRLSDVSAVTADSVKGRFTISTDNSKNTLYLQMNSLRAEDTAVYYCTASRSPSGIRYYKPDYWGQGTLVTVSSGGGGSQSQLVESGGGLVKPGGSLRLSCVASGFTISRSIMSWYRQAPGKERDWVASIGSAGNTNYVDSVKGRFTISRDNAKNSLYLQMNSLRAEDTAVYYCKTTLAVSFSEYWGQGTLVTVSSGGGGSGGGGSQSQLVESGGGLVKPGGSLRLSCVASGFTISRSIMSWYRQAPGKERDWVASIGSAGNTNYVDSVKGRFTISRDNAKNSLYLQMNSLRAEDTAVYYCKTTLAVSFSEYWGQGTLVTVSSGGGGSEVQLVESGGGLVQPGNSLRLSCAASGFTFSSFGMSWVRQAPGKGLEWVSSISGSGSDTLYADSVKGRFTISRDNAKTTLYLQMNSLRPEDTAVYYCTIGGSLSRSSQGTLVTVSS

SEQ ID NO: 78 - protein, 486 aa, synthetic construct
EVQLVESGGGLVQPGGSLRLSCSASGTIIGTYTMAWYRQAPGKQREMVAIITPGGGSHHADSVKGRFTISRDNSKNTLYLQMSSLRAEDTAVYYCNAKARWGTTEYWGQGTLVTVSSGGGGSEVQLVESGGGLVQPGGSLRLSCTASGNIFSSYHMGWFRQAPGKQREFIAYITTREITNYADSVKGRFTISRDNSKNTLYLQMNSLRAEDTAVYYCIADQSREIRRSWGQGTLVTVSSGGGGSGGGGSQSQLVESGGGLVKPGGSLRLSCVASGFTISRSIMSWYRQAPGKERDWVASIGSAGNTNYVDSVKGRFTISRDNAKNSLYLQMNSLRAEDTAVYYCKTTLAVSFSEYWGQGTLVTVSSGGGGSEVQLVESGGGLVQPGNSLRLSCAASGFTFSSFGMSWVRQAPGKGLEWVSSISGSGSDTLYADSVKGRFTISRDNAKTTLYLQMNSLRPEDTAVYYCTIGGSLSRSSQGTLVTVSS

SEQ ID NO: 79 - protein, 486 aa, synthetic construct
EVQLVESGGGLVQPGGSLRLSCSASGTIIGTYTMAWYRQAPGKQREMVAIITPGGGSHHADSVKGRFTISRDNSKNTLYLQMSSLRAEDTAVYYCNAKARWGTTEYWGQGTLVTVSSGGGGSEVQLVESGGGLVQPGGSLRLSCTASGNIFSSYHMGWFRQAPGKQREFIAYITTREITNYADSVKGRFTISRDNSKNTLYLQMNSLRAEDTAVYYCIADQSREIRRSWGQGTLVTVSSGGGGSGGGGSEVQLVESGGGLVQPGGSLRLSCTASGNIFSSYHMGWFRQAPGKQREFIAYITTREITNYADSVKGRFTISRDNSKNTLYLQMNSLRAEDTAVYYCIADQSREIRRSWGQGTLVTVSSGGGGSEVQLVESGGGLVQPGNSLRLSCAASGFTFSSFGMSWVRQAPGKGLEWVSSISGSGSDTLYADSVKGRFTISRDNAKTTLYLQMNSLRPEDTAVYYCTIGGSLSRSSQGTLVTVSS

SEQ ID NO: 80 - protein, 486 aa, synthetic construct
EVQLVESGGGLVQPGGSLRLSCSASGTIIGTYTMAWYRQAPGKQREMVAIITPGGGSHHADSVKGRFTISRDNSKNTLYLQMSSLRAEDTAVYYCNAKARWGTTEYWGQGTLVTVSSGGGGSQSQLVESGGGLVKPGGSLRLSCVASGFTISRSIMSWYRQAPGKERDWVASIGSAGNTNYVDSVKGRFTISRDNAKNSLYLQMNSLRAEDTAVYYCKTTLAVSFSEYWGQGTLVTVSSGGGGSGGGGSQSQLVESGGGLVKPGGSLRLSCVASGFTISRSIMSWYRQAPGKERDWVASIGSAGNTNYVDSVKGRFTISRDNAKNSLYLQMNSLRAEDTAVYYCKTTLAVSFSEYWGQGTLVTVSSGGGGSEVQLVESGGGLVQPGNSLRLSCAASGFTFSSFGMSWVRQAPGKGLEWVSSISGSGSDTLYADSVKGRFTISRDNAKTTLYLQMNSLRPEDTAVYYCTIGGSLSRSSQGTLVTVSS

SEQ ID NO: 81 - protein, 495 aa, synthetic construct
EVQLLESGGGLVQPGGSLRLSCAASGLTFSYYAMAWFRQAPGKEREFVAAINWNQGNTYNTDSVKGRFTISRDNSKNTVYLQMNSLTPEDTAVYYCAVRYNQASYLVARSSDYNYWGQGTLVTVSSGGGGSEVQLVESGGGLVQPGGSLRLSCTASGNIFSSYHMGWFRQAPGKQREFIAYITTREITNYADSVKGRFTISRDNSKNTLYLQMNSLRAEDTAVYYCIADQSREIRRSWGQGTLVTVSSGGGGSGGGGSQSQLVESGGGLVKPGGSLRLSCVASGFTISRSIMSWYRQAPGKERDWVASIGSAGNTNYVDSVKGRFTISRDNAKNSLYLQMNSLRAEDTAVYYCKTTLAVSFSEYWGQGTLVTVSSGGGGSEVQLVESGGGLVQPGNSLRLSCAASGFTFSSFGMSWVRQAPGKGLEWVSSISGSGSDTLYADSVKGRFTISRDNAKTTLYLQMNSLRPEDTAVYYCTIGGSLSRSSQGTLVTVSS

SEQ ID NO: 82 - protein, 495 aa, synthetic construct
EVQLLESGGGLVQPGGSLRLSCAASGLTFSYYAMAWFRQAPGKEREFVAAINWNQGNTYNTDSVKGRFTISRDNSKNTVYLQMNSLTPEDTAVYYCAVRYNQASYLVARSSDYNYWGQGTLVTVSSGGGGSEVQLVESGGGLVQPGGSLRLSCTASGNIFSSYHMGWFRQAPGKQREFIAYITTREITNYADSVKGRFTISRDNSKNTLYLQMNSLRAEDTAVYYCIADQSREIRRSWGQGTLVTVSSGGGGSGGGGSEVQLVESGGGLVQPGGSLRLSCTASGNIFSSYHMGWFRQAPGKQREFIAYITTREITNYADSVKGRFTISRDNSKNTLYLQMNSLRAEDTAVYYCIADQSREIRRSWGQGTLVTVSSGGGGSEVQLVESGGGLVQPGNSLRLSCAASGFTFSSFGMSWVRQAPGKGLEWVSSISGSGSDTLYADSVKGRFTISRDNAKTTLYLQMNSLRPEDTAVYYCTIGGSLSRSSQGTLVTVSS

SEQ ID NO: 83 - protein, 495 aa, synthetic construct
EVQLLESGGGLVQPGGSLRLSCAASGLTFSYYAMAWFRQAPGKEREFVAAINWNQGNTYNTDSVKGRFTISRDNSKNTVYLQMNSLTPEDTAVYYCAVRYNQASYLVARSSDYNYWGQGTLVTVSSGGGGSQSQLVESGGGLVKPGGSLRLSCVASGFTISRSIMSWYRQAPGKERDWVASIGSAGNTNYVDSVKGRFTISRDNAKNSLYLQMNSLRAEDTAVYYCKTTLAVSFSEYWGQGTLVTVSSGGGGSGGGGSQSQLVESGGGLVKPGGSLRLSCVASGFTISRSIMSWYRQAPGKERDWVASIGSAGNTNYVDSVKGRFTISRDNAKNSLYLQMNSLRAEDTAVYYCKTTLAVSFSEYWGQGTLVTVSSGGGGSEVQLVESGGGLVQPGNSLRLSCAASGFTFSSFGMSWVRQAPGKGLEWVSSISGSGSDTLYADSVKGRFTISRDNAKTTLYLQMNSLRPEDTAVYYCTIGGSLSRSSQGTLVTVSS

SEQ ID NO: 84 - protein, 123 aa, synthetic construct
QVQLVESGGGLVQPGGSLRLSCAASGRTGSLHAMGWFRQAPGKERERVATLQLSDVSAVTADSVKGRFTISTDNSKNSVYLQMNSLRAEDTAVYYCTASRSPSGIRYYKPDYWGQGTLVTVSS

SEQ ID NO: 85 - protein, 17 aa, synthetic construct
TLQLSDVSAVTADSVKG

SEQ ID NO: 86 - protein, 355 aa, synthetic construct
QVQLVESGGGLVQPGGSLRLSCAASGRTGSLHAMGWFRQAPGKERERVATLQLSDVSAVTADSVKGRFTISTDNSKNSVYLQMNSLRAEDTAVYYCTASRSPSGIRYYKPDYWGQGTLVTVSSEPKSSDKTHTCPPCPAPEAAGGPSVFLFPPKPKDTLMISRTPEVTCVVVDVSHEDPEVKFNWYVDGVEVHNAKTKPREEQYNSTYRVVSVLTVLHQDWLNGKEYKCKVSNKALPAPIEKTISKAKGQPREPQVYTLPPSRDELTKNQVSLSCAVKGFYPSDIAVEWESNGQPENNYKTTPPVLDSDGSFFLVSKLTVDKSRWQQGNVFSCSVMHEALHNHYTQKSLSLSPGK

SEQ ID NO: 87 - protein, 476 aa, synthetic construct
QSQLAESGGGLVQSGGSLGLSCVASGFTISRSIMSWYRQPPGKERDWVASIGSAGNTNYVDSVKGRFTISRDVAKNTVYLQMNSLKPEDTAVYYCKTTLAVSFSEYWGQGTQVTVSSGGGGSGGGGSEVQLVESGGGLIQAGGSLRLSCTASGNIFSSYHMGWFRQAPGKQREFIAYITTREITNYADSVKGRFTISRDNSKNTVYLQMNNLRSEDTAVYYCIADQSREIRRSWGQGTLVTVSSEPKSSDKTHTCPPCPAPEAAGGPSVFLFPPKPKDTLMISRTPEVTCVVVDVSHEDPEVKFNWYVDGVEVHNAKTKPREEQYNSTYRVVSVLTVLHQDWLNGKEYKCKVSNKALPAPIEKTISKAKGQPREPQVYTLPPSRDELTKNQVSLWCLVKGFYPSDIAVEWESNGQPENNYKTTPPVLDSDGSFFLYSKLTVDKSRWQQGNVFSCSVMHEALHNHYTQKSLSLSPGK

SEQ ID NO: 88 - protein, 349 aa, synthetic construct
QSQLAESGGGLVQSGGSLGLSCVASGFTISRSIMSWYRQPPGKERDWVASIGSAGNTNYVDSVKGRFTISRDVAKNTVYLQMNSLKPEDTAVYYCKTTLAVSFSEYWGQGTQVTVSSEPKSSDKTHTCPPCPAPELLGGPSVFLFPPKPKDTLMISRTPEVTCVVVDVSHEDPEVKFNWYVDGVEVHNAKTKPREEQYNSTYRVVSVLTVLHQDWLNGKEYKCKVSNKALPAPIEKTISKAKGQPREPQVCTLPPSRDELTKNQVSLSCAVKGFYPSDIAVEWESNGQPENNYKTTPPVLDSDGSFFLVSKLTVDKSRWQQGNVFSCSVMHEALHNHYTQKSLSLSPGK

SEQ ID NO: 89 - protein, 349 aa, synthetic construct
EVQLVESGGGLIQAGGSLRLSCTASGNIFSSYHMGWFRQAPGKQREFIAYITTREITNYADSVKGRFTISRDNSKNTVYLQMNNLRSEDTAVYYCIADQSREIRRSWGQGTLVTVSSEPKSSDKTHTCPPCPAPELLGGPSVFLFPPKPKDTLMISRTPEVTCVVVDVSHEDPEVKFNWYVDGVEVHNAKTKPREEQYNSTYRVVSVLTVLHQDWLNGKEYKCKVSNKALPAPIEKTISKAKGQPREPQVYTLPPCRDELTKNQVSLWCLVKGFYPSDIAVEWESNGQPENNYKTTPPVLDSDGSFFLYSKLTVDKSRWQQGNVFSCSVMHEALHNHYTQKSLSLSPGK

SEQ ID NO: 90 - protein, 349 aa, synthetic construct
QSQLAESGGGLVQSGGSLGLSCVASGFTISRSIMSWYRQPPGKERDWVASIGSAGNTNYVDSVKGRFTISRDVAKNTVYLQMNSLKPEDTAVYYCKTTLAVSFSEYWGQGTQVTVSSEPKSSDKTHTCPPCPAPELLGGPSVFLFPPKPKDTLMISRTPEVTCVVVDVSHEDPEVKFNWYVDGVEVHNAKTKPREEQYNSTYRVVSVLTVLHQDWLNGKEYKCKVSNKALPAPIEKTISKAKGQPREPQVYTLPPSRDELTKNQVSLTCLVKGFYPSDIAVEWESNGQPENNYKTTPPVLDSDGSFFLYSKLTVDKSRWQQGNVFSCSVMHEALHNHYTQKSLSLSPGK

SEQ ID NO: 91 - protein, 349 aa, synthetic construct
EVQLVESGGGLIQAGGSLRLSCTASGNIFSSYHMGWFRQAPGKQREFIAYITTREITNYADSVKGRFTISRDNSKNTVYLQMNNLRSEDTAVYYCIADQSREIRRSWGQGTLVTVSSEPKSSDKTHTCPPCPAPELLGGPSVFLFPPKPKDTLMISRTPEVTCVVVDVSHEDPEVKFNWYVDGVEVHNAKTKPREEQYNSTYRVVSVLTVLHQDWLNGKEYKCKVSNKALPAPIEKTISKAKGQPREPQVYTLPPSRDELTKNQVSLTCLVKGFYPSDIAVEWESNGQPENNYKTTPPVLDSDGSFFLYSKLTVDKSRWQQGNVFSCSVMHEALHNHYTQKSLSLSPGK

SEQ ID NO: 92 - protein, 347 aa, synthetic construct
AVQLVDSGGGLVQPGGSLRLSCAASGFAFNIYNMGWYRQAPGKQRELVATIAADGSTGYADSVKGRFTISRDNVKNKVDLQMNSLKPEDTAVYYCKRELGPFSSWGQGTQVTVSSEPKSSDKTHTCPPCPAPEAAGGPSVFLFPPKPKDTLMISRTPEVTCVVVDVSHEDPEVKFNWYVDGVEVHNAKTKPREEQYNSTYRVVSVLTVLHQDWLNGKEYKCKVSNKALPAPIEKTISKAKGQPREPQVYTLPPSRDELTKNQVSLSCAVKGFYPSDIAVEWESNGQPENNYKTTPPVLDSDGSFFLVSKLTVDKSRWQQGNVFSCSVMHEALHNHYTQKSLSLSPGK

SEQ ID NO: 93 - protein, 472 aa, synthetic construct
AVQLVDSGGGLVQPGGSLRLSCAASGFAFNIYNMGWYRQAPGKQRELVATIAADGSTGYADSVKGRFTISRDNVKNKVDLQMNSLKPEDTAVYYCKRELGPFSSWGQGTQVTVSSGGGGSGGGGSAVQLVDSGGGLVQPGGSLRLSCAASGFAFNIYNMGWYRQAPGKQRELVATIAADGSTGYADSVKGRFTISRDNVKNKVDLQMNSLKPEDTAVYYCKRELGPFSSWGQGTQVTVSSEPKSSDKTHTCPPCPAPEAAGGPSVFLFPPKPKDTLMISRTPEVTCVVVDVSHEDPEVKFNWYVDGVEVHNAKTKPREEQYNSTYRVVSVLTVLHQDWLNGKEYKCKVSNKALPAPIEKTISKAKGQPREPQVYTLPPSRDELTKNQVSLWCLVKGFYPSDIAVEWESNGQPENNYKTTPPVLDSDGSFFLYSKLTVDKSRWQQGNVFSCSVMHEALHNHYTQKSLSLSPGK

SEQ ID NO: 94 - protein, 117 aa, synthetic construct
EVQLVESGGGLVQPGGSLRLSCAASGTIIGTYTMAWYRQAPGKQREMVAIITPGGGSHHADSVKGRFTISRDNSKNTLYLQMNSLRAEDTAVYYCNAKARWGTTEYWGQGTMVTVSS

SEQ ID NO: 95 - protein, 117 aa, synthetic construct
EVQLVESGGGLVQPGGSLRLSCAASGTIIGTYTMAWYRQAPGKQREMVAIITPGGGSHHADSVKGRFTISRDNSKNTVYLQMNSLRAEDTAVYYCNAKARWGTTEYWGQGTMVTVSS

SEQ ID NO: 96 - protein, 117 aa, synthetic construct
EVQLVESGGGLVQPGGSLRLSCSASGTIIGTYTMAWYRQAPGKQREMVAIITPGGGSHHADSVKGRFTISRDNSKSTVYLQMSSLRAEDTAVYYCNAKARWGTTEYWGQGTLVTVSS

SEQ ID NO: 97 - protein, 117 aa, synthetic construct
EVQLVESGGGLVQPGGSLRLSCSASGTIIGTYTMAWYRQAPGKQREMVAIITPGGGSHHADSVKGRFTISRDNGKNTLYLQMSSLRAEDTAVYYCNAKARWGTTEYWGQGTLVTVSS

SEQ ID NO: 98 - protein, 117 aa, synthetic construct
EVQLVESGGGLVQPGGSLRLSCSASGTIIGTYTMAWYRQAPGKQREMVAIITPGGGSHHADSVKGRFTISRDNSKNTLYLQMSSLRFEDTAVYYCNAKARWGTTEYWGQGTLVTVSS

SEQ ID NO: 99 - protein, 117 aa, synthetic construct
EVQLVESGGGLVQPGGSLRLDCSASGTIIGTYTMAWYRQAPGKQREMVAIITPGGGSHHADSVKGRFTISRDNSKSTVYLQMSSLRFEDTAVYYCNAKARWGTTEYWGQGTLVTVSS

SEQ ID NO: 100 - protein, 126 aa, synthetic construct
EVQLLESGGGLVQPGGSLRLSCAASGLTFSYYAMAWFRQAPGKEREFVAAINWNGGNTYNTDSVKGRFTISRDNSKNTVYLQMNSLTPEDTAVYYCAVRYNSASYLVARSSDYNYWGQGTLVTVSS

SEQ ID NO: 101 - protein, 126 aa, synthetic construct
EVQLLESGGGLVQPGGSLRLSCAASGLTFSYYAMAWFRQAPGKEREFVAAINWNGGNTYNTDSVKGRFTISRDNSKNTVYLQMNSLRSEDTAVYYCAVRYNSASYLVARSSDYNYWGQGTLVTVSS

SEQ ID NO: 102 - protein, 126 aa, synthetic construct
EVQLLESGGGLVQPGGSLRLSCAASGLTFSYYAMAWFRQAPGKEREFVAAINWNAGNTYNTDSVKGRFTISRDNSKNTVYLQMNSLTPEDTAVYYCAVRYNAASYLVARSSDYNYWGQGTLVTVSS

SEQ ID NO: 103 - protein, 17 aa, synthetic construct
AINWNAGNTYNTDSVKG

SEQ ID NO: 104 - protein, 17 aa, synthetic construct
RYNAASYLVARSSDYNY

SEQ ID NO: 105 - protein, 123 aa, synthetic construct
QVQLVQSGPEVKKPGTSVKVSCKASGRTGSLHAMGWFRQARGQERERVATLNLSDGSAVTADSVKGRFTITTDNSKNSVYMELSSLRSEDTAVYYCTASRSPSGIRYYKPDYWGQGTMVTVSS

SEQ ID NO: 106 - protein, 123 aa, synthetic construct
QVQLVESGGGLVQPGGSLRLSCAASGRTGSLHAMGWFRQAPGKERERVATLNLSDGSAVTADSVKGRFTISTDNSKNSVYLQMNSLRAEDTAVYYCTASRSPSGIRYYKPDYWGQGTLVTVSS

SEQ ID NO: 107 - protein, 123 aa, synthetic construct
QVQLVESGGGLVQAGGSLRLSCAASGRTGSLHAMGWFRQAPGKERERVATLQLSDGSAVTADSVKGRFTISTDNTKNSVYLQMNSLKPEDTAVYYCTASRSPSGIRYYKPDYWGQGTQVTVSS

SEQ ID NO: 108 - protein, 123 aa, synthetic construct
QVQLVESGGGLVQAGGSLRLSCAASGRTGSLHAMGWFRQAPGKERERVATLNLADGSAVTADSVKGRFTISTDNTKNSVYLQMNSLKPEDTAVYYCTASRSPSGIRYYKPDYWGQGTQVTVSS

SEQ ID NO: 109 - protein, 123 aa, synthetic construct
QVQLVESGGGLVQAGGSLRLSCAASGRTGSLHAMGWFRQAPGKERERVATLQLTDGSAVTADSVKGRFTISTDNTKNSVYLQMNSLKPEDTAVYYCTASRSPSGIRYYKPDYWGQGTQVTVSS

SEQ ID NO: 110 - protein, 123 aa, synthetic construct
QVQLVESGGGLVQAGGSLRLSCAASGRTGSLHAMGWFRQAPGKERERVATLNLSEGSAVTADSVKGRFTISTDNTKNSVYLQMNSLKPEDTAVYYCTASRSPSGIRYYKPDYWGQGTQVTVSS

SEQ ID NO: 111 - protein, 123 aa, synthetic construct
QVQLVESGGGLVQAGGSLRLSCAASGRTGSLHAMGWFRQAPGKERERVATLNLSDVSAVTADSVKGRFTISTDNTKNSVYLQMNSLKPEDTAVYYCTASRSPSGIRYYKPDYWGQGTQVTVSS

SEQ ID NO: 112 - protein, 123 aa, synthetic construct
QVQLVESGGGLVQAGGSLRLSCAASGRTGSLHAMGWFRQAPGKERERVATLNLSDASAVTADSVKGRFTISTDNTKNSVYLQMNSLKPEDTAVYYCTASRSPSGIRYYKPDYWGQGTQVTVSS

SEQ ID NO: 113 - protein, 123 aa, synthetic construct
QVQLVESGGGLVQPGGSLRLSCAASGRTGSLHAMGWFRQAPGKERERVATLNLSDVSAVTADSVKGRFTISTDNSKNSVYLQMNSLRAEDTAVYYCTASRSPSGIRYYKPDYWGQGTLVTVSS

SEQ ID NO: 114 - protein, 123 aa, synthetic construct
QVQLVESGGGLVQPGGSLRLSCAASGRTGSLHAMGWFRQAPGKERERVATLRLSDVSAVTADSVKGRFTISTDNSKNSVYLQMNSLRAEDTAVYYCTASRSPSGIRYYKPDYWGQGTLVTVSS

SEQ ID NO: 115 - protein, 17 aa, synthetic construct
TLQLSDGSAVTADSVKG

SEQ ID NO: 116 - protein, 17 aa, synthetic construct
TLNLADGSAVTADSVKG

SEQ ID NO: 117 - protein, 17 aa, synthetic construct
TLQLTDGSAVTADSVKG

SEQ ID NO: 118 - protein, 17 aa, synthetic construct
TLNLSEGSAVTADSVKG

SEQ ID NO: 119 - protein, 17 aa, synthetic construct
TLNLSDVSAVTADSVKG

SEQ ID NO: 120 - protein, 17 aa, synthetic construct
TLNLSDASAVTADSVKG

SEQ ID NO: 121 - protein, 117 aa, synthetic construct
EVQLVESGGGLVQPGGSLRLSCAASGNIFSSNHMGWVRQAPGKGLEWVAYITTREITNYADSVKGRFTISRDNSKNTVYLQMNSLRAEDTAVYYCIADQSREIRRSWGQGTLVTVSS

SEQ ID NO: 122 - protein, 117 aa, synthetic construct
EVQLVESGGGLIQPGGSLRLSCKASGNIFSSNHMGWFRQAPGKQLEWVAYITTREITNYADSVKGRFTISRDNSKNTVYLQMNNLRSEDTAVYYCIADQSREIRRSWGQGTLVTVSS

SEQ ID NO: 123 - protein, 117 aa, synthetic construct
EVQLVESGGGLIQPGGSLRLSCTASGNIFSSNHMGWFRQAPGKQLEWIAYITTREITNYADSVKGRFTISRDNSKNTVYLQMNNLRSEDTAVYYCIADQSREIRRSWGQGTQVTVSS

SEQ ID NO: 124 - protein, 117 aa, synthetic construct
EVQLVESGGGLIQAGGSLRLSCTASGNIFSSNHMGWFRQAPGKQREFIAYITTREITNYADSVKGRFTISRDNSKNTVYLQMNNLRSEDTAVYYCIADQSREIRRSWGQGTLVTVSS

SEQ ID NO: 125 - protein, 117 aa, synthetic construct
EVQLVESGGGLVQAGGSLRLSCVASGNIFSSYHMGWFRQAPGKQREFIAYITTREITNYADSVKGRFTISRDNTKNTVYLQMNVLKPEDTAVYYCIADQSREIRRSWGQGTQVTVSS

SEQ ID NO: 126 - protein, 117 aa, synthetic construct
EVQLVESGGGLVQAGGSLRLSCVASGNIFSSHHMGWFRQAPGKQREFIAYITTREITNYADSVKGRFTISRDNTKNTVYLQMNVLKPEDTAVYYCIADQSREIRRSWGQGTQVTVSS

SEQ ID NO: 127 - protein, 117 aa, synthetic construct
EVQLVESGGGLVQAGGSLRLSCVASGNIFSSFHMGWFRQAPGKQREFIAYITTREITNYADSVKGRFTISRDNTKNTVYLQMNVLKPEDTAVYYCIADQSREIRRSWGQGTQVTVSS

SEQ ID NO: 128 - protein, 117 aa, synthetic construct
EVQLVESGGGLVQAGGSLRLSCVASGNIFSSDHMGWFRQAPGKQREFIAYITTREITNYADSVKGRFTISRDNTKNTVYLQMNVLKPEDTAVYYCIADQSREIRRSWGQGTQVTVSS

SEQ ID NO: 129 - protein, 117 aa, synthetic construct
EVQLVESGGGLIQAGGSLRLSCTASGNIFSSYHMGWFRQAPGKQREFIAYITTREITNYADSVKGRFTISRDNSKNTLYLQMNSLRAEDTAVYYCIADQSREIRRSWGQGTLVTVSS

SEQ ID NO: 130 - protein, 117 aa, synthetic construct
EVQLVESGGGLIQAGGSLRLSCTASGNIFSSYHMGWFRQAPGKQREFIAYITTREITNYADSVKGRFTISRDNAKNTVYLQMNSLRPEDTAVYYCIADQSREIRRSWGQGTLVTVSS

SEQ ID NO: 131 - protein, 5 aa, synthetic construct
SHHMG

SEQ ID NO: 132 - protein, 5 aa, synthetic construct
SFHMG

SEQ ID NO: 133 - protein, 5 aa, synthetic construct
SDHMG

SEQ ID NO: 134 - protein, 117 aa, synthetic construct
ESQLLESGGGLVQPGGSLRLSCVASGFTISRSIMSWYRQAPGKERDWVASIGSAGNTNYVDSVKGRFTISRDNSKNTVYLQMNSLRAEDTAVYYCKTTLAVSFSEYWGQGTLVTVSS

SEQ ID NO: 135 - protein, 117 aa, synthetic construct
ESQLLESGGGLVQPGGSLRLSCVASGFTISRSIMSWYRQAPGKERDWVASIGSAGNTNYVDSVKGRFTISRDVSKNTLYLQMNSLRAEDTAVYYCKTTLAVSFSEYWGQGTLVTVSS

SEQ ID NO: 136 - protein, 117 aa, synthetic construct
QSQLVESGGGLVKPGGSLRLSCVASGFTISRSIMSWYRQPPGKERDWVASIGSAGNTNYVDSVKGRFTISRDNAKNSLYLQMNSLRAEDTAVYYCKTTLAVSFSEYWGQGTLVTVSS

SEQ ID NO: 137 - protein, 232 aa, synthetic construct
EPKSSDKTHTCPPCPAPEAAGGPSVFLFPPKPKDTLMISRTPEVTCVVVDVSHEDPEVKFNWYVDGVEVHNAKTKPREEQYNSTYRVVSVLTVLHQDWLNGKEYKCKVSNKALPAPIEKTISKAKGQPREPQVYTLPPSRDELTKNQVSLSCAVKGFYPSDIAVEWESNGQPENNYKTTPPVLDSDGSFFLVSKLTVDKSRWQQGNVFSCSVMHEALHNHYTQKSLSLSPGK

SEQ ID NO: 138 - protein, 232 aa, synthetic construct
EPKSSDKTHTCPPCPAPEAAGGPSVFLFPPKPKDTLMISRTPEVTCVVVDVSHEDPEVKFNWYVDGVEVHNAKTKPREEQYNSTYRVVSVLTVLHQDWLNGKEYKCKVSNKALPAPIEKTISKAKGQPREPQVYTLPPSRDELTKNQVSLWCLVKGFYPSDIAVEWESNGQPENNYKTTPPVLDSDGSFFLYSKLTVDKSRWQQGNVFSCSVMHEALHNHYTQKSLSLSPGK